European Patent Specification EP 3 183 580 B1, published March 26, 2025. Title: HOMOGENOUS THERMAL SHIFT LIGAND BINDING ASSAY. Applicant: THE BOARD OF TRUSTEES OF THE LELAND STANFORD JUNIOR UNIVERSITY Treiber, Daniel K Menichelli, Elena. The sequence listing filed with the application follows.

SEQUENCE LISTING (4 sequences)

SEQ ID NO: 1 - protein, 52 aa, E. coli
  PEPTIDE (1)..(52): Wild-type ED
MGVITDSLAVVLQRRDWENPGVTQLNRLAAHPPFASWRNSEEARTDRPSQQL

SEQ ID NO: 2 - protein, 42 aa, E. coli
  PEPTIDE (1)..(42): Prolabel ED
NSLAVVLQRRDWENPGVTQLNRLAAHPPFASWRNSEEARTDR

SEQ ID NO: 3 - protein, 52 aa, E. coli
  PEPTIDE (1)..(52): W34Y ED
MGVITDSLAVVLQRRDWENPGVTQLNRLAAHPPFASYRNSEEARTDRPSQQL

SEQ ID NO: 4 - protein, 42 aa, E. coli; identical to SEQ ID NO: 2
  PEPTIDE (1)..(42): Enhanced Prolabel ED